European Patent Specification EP 4 326 861 B1, published December 17, 2025. Title: ENGINEERED MEGANUCLEASES THAT TARGET HUMAN MITOCHONDRIAL GENOMES. Applicant: Moraes, Carlos Smith, James J. Tomberlin, Ginger Morris, John Shoop, Wendy. The sequence listing filed with the application follows.

SEQUENCE LISTING (72 sequences)

SEQ ID NO: 1 - DNA, 22 bp, Homo sapiens
cagggcccggtaatcgcataaa

SEQ ID NO: 2 - DNA, 22 bp, Homo sapiens
gtcccgggccattagcgtattt

SEQ ID NO: 3 - protein, 354 aa, Artificial Sequence
  Synthesized
MNTKYNKEFLLYLAGFVDSDGSIFARIEPTQSAKFKHKLRLTFRVHQKTQRRWFLDKLVDEIGVGYVYDTGSVSDYTLSQIKPLHNFLTQLQPFLKLKQKQANLVLKIIEQLPSAKESPDKFLEVCTWVDQIAALNDSKTRKTTSETVRAVLDSLPGSVGGLSPSQASSAASSASSSPGSGISEALRAGAGSGTGYNKEFLLYLAGFVDGDGSIYACILPNQGSKFKHALQLFFTVGQKTCRRWFLDKLVDEIGVGYVHDHGTISQYRLSEIKPLHNFLTQLQPFLKLKQKQANLVLKIIEQLPSAKESPDKFLEVCTWVDQIAALNDSRTRKTTSETVRAVLDSLSEKKKSSP

SEQ ID NO: 4 - protein, 354 aa, Artificial Sequence
  Synthesized
MNTKYNKEFLLYLAGFVDADGSIFARIEPTQSAKFKHKLRLTFRVHQKTQRRWFLDKLVDEIGVGYVYDTGSVSDYTLSEIKPLHNFLTQLQPFLKLKQKQANLVLKIIEQLPSAKESPDKFLEVCTWVDQIAALNDSKTRKTTSETVRAVLDSLPGSVGGLSPSQASSAASSASSSPGSGISEALRAGAGSGTGYNKEFLLYLAGFVDGDGSIYACILPNQGSKFKHALQLFFTVGQKTCRRWFLDKLVDEIGVGYVNDFGSISQYRLSEIKPLYNFLTQLQPFLKLKQKQANLVLKIIEQLPSAKESPDKFLEVCTWVDQIAALNDSRTRKTTSETVRAVLDSLSEKKKSSP

SEQ ID NO: 5 - protein, 354 aa, Artificial Sequence
  Synthesized
MNTKYNKEFLLYLAGFVDADGSIFARIEPTQSAKFKHKLRLTFRVHQKTQRRWFLDKLVDEIGVGYVYDTGSVSDYTLSQIKPLHNFLTQLQPFLKLKQKQANLVLKIIEQLPSAKESPDKFLEVCTWVDQIAALNDSKTRKTTSETVRAVLDSLPGSVGGLSPSQASSAASSASSSPGSGISEALRAGAGSGTGYNKEFLLYLAGFVDGDGSIYACILPNQGSKFKHALQLFFTVGQKTCRRWFLDKLVDEIGVGYVHDFGLISQYRLSEIKPLHNFLTQLQPFLKLKQKQANLVLKIIEQLPSAKESPDKFLEVCTWVDQIAALNDSRTRKTTSETVRAVLDSLSEKKKSSP

SEQ ID NO: 6 - protein, 354 aa, Artificial Sequence
  Synthesized
MNTKYNKEFLLYLAGFVDADGSIFARIEPTQSAKFKHKLRLTFRVHQKTQRRWFLDKLVDEIGVGYVYDTGSVSDYTLSEIKPLHNFLTQLQPFLKLKQKQANLVLKIIEQLPSAKESPDKFLEVCTWVDQIAALNDSKTRKTTSETVRAVLDSLPGSVGGLSPSQASSAASSASSSPGSGISEAPRAGAGSGTGYNKEFLLYLAGFVDGDGSIYACILPNQGSKFKHALQLFFTVGQKTCRRWFLDKLVDEIGVGYVHDHGLIAQYRLSEIKPLHNFLTQLQPFLKLKQKQANLVLKIIEQLPSAKESPDKFLEVCTWVDQIAALNDSRTRKTTSETVRAVLDSLSEKKKSSP

SEQ ID NO: 7 - protein, 354 aa, Artificial Sequence
  Synthesized
MNTKYNKEFLLYLAGFVDADGSIFARIEPTQSAKFKHKLRLTFRVHQKTQRRWFLDKLVDEIGVGYVYDTGSVSDYTLSQIKPLHNFLTQLQPFLKLKQKQANLVLKIIEQLPSAKESPDKFLEVCTWVDQIAALNDSKTRKTTSETVRAVLDSLPGSVGGLSPSQASSAASSASSSPGSGISEALRAGAGSGTGYNKEFLLYLAGFVDGDGSIYACILPNQGSKFKHALQLFFTVGQKTCRRWFLDKLVDEIGVGYVNDFGPVSQYRLSEIKPLHNFLTQLQPFLKLKQKQANLVLKIIEQLPSAKESPDKFLEVCTWVDQIAALNDSRTRKTTSETVRAVLDSLSEKKKSSP

SEQ ID NO: 8 - protein, 354 aa, Artificial Sequence
  Synthesized
MNTKYNKEFLLYLAGFVDADGSIFARIEPTQSAKFKHKLRLTFRVWQKTQRRWFLDKLVDEIGVGYVYDEGSVSSYTLSEIKPLHNFLTQLQPFLKLKQKQANLVLKIIEQLPSAKESPDKFLEVCTWVDQIAALNDSKTRKTTSETVRAVLDSLPGSVGGLSPSQASSAASSASSSPGSGISEALRAGAGSGTGYNKEFLLYLAGFVDGDGSIYACILPNQGSKFKHALQLFFTVGQKTCRRWFLDKLVDEIGVGYVQDHGRISQYRLSEIKPLHNFLTQLQPFLKLKQKQANLVLKIIEQLPSAKESPDKFLEVCTWVDQIAALNDSRTRKTTSETVRAVLDSLSEKKKSSP

SEQ ID NO: 9 - protein, 354 aa, Artificial Sequence
  Synthesized
MNTKYNKEFLLYLAGFVDSDGSIFARIEPTQSAKFKHKLRLTFRVHQKTQRRWFLDKLVDEIGVGYVYDTGSVSDYTLSQIKPLHNFLTQLQPFLKLKQKQANLVLKIIEQLPSAKESPDKFLEVCTWVDQIAALNDSKTRKTTSETVRAVLDSLPGSVGGLSPSQASSAASSASSSPGSGISEALRAGAGSGTGYNKEFLLYLAGFVDGDGSIYACILPNQGSKFKHALQLFFTVGQKTCRRWFLDKLVDEIGVGYVQDHGTISQYRLSEIKPLHNFLTQLQPFLKLKQKQANLVLKIIEQLPSAKESPDKFLEVCTWVDQIAALNDSRTRKTTSETVRAVLDSLSEKKKSSP

SEQ ID NO: 10 - protein, 354 aa, Artificial Sequence
  Synthesized
MNTKYNKEFLLYLAGFVDSDGSIFARIEPTQSAKFKHKLRLTFRVWQKTQRRWFLDKLVDEIGVGYVYDEGSVSSYTLSEIKPLHNFLTQLQPFLKLKQKQANLVLKIIEQLPSAKESPDKFLEVCTWVDQIAALNDSKTRKTTSETVRAVLDSLPGSVGGLSPSQASSAASSASSSPGSGISEALRAGAGSGTGYNKEFLLYLAGFVDGDGSIYACILPNQGSKFKHALQLFFTVGQKTCRRWFLDKLVDEIGVGYVQDHGRISQYRLSEIKPLHNFLTQLQPFLKLKQKQANLVLKIIEQLPSAKESPDKFLEVCTWVDQIAALNDSRTRKTTSETVRAVLDSLSEKKKSSP

SEQ ID NO: 11 - protein, 354 aa, Artificial Sequence
  Synthesized
MNTKYNKEFLLYLAGFVDSDGSIFARIEPTQSAKFKHKLRLTFRVHQKTQRRWFLDKLVDEIGVGYVYDTGSVSDYTLSQIKPLHNFLTQLQPFLKLKQKQANLVLKIIEQLPSAKESPDKFLEVCTWVDQIAALNDSKTRKTTSETVRAVLDSLPGSVGGLSPSQASSAASSASSSPGSGISEALRAGAGSGTGYNKEFLLYLAGFVDGDGSIYACILPNQGSKFKHALQLFFTVGQKTCRRWFLDKLVDEIGVGYVHDHGRISQYRLSEIKPLHNFLTQLQPFLKLKQKQANLVLKIIEQLPSAKESPDKFLEVCTWVDQIAALNDSRTRKTTSETVRAVLDSLSEKKKSSP

SEQ ID NO: 12 - protein, 354 aa, Artificial Sequence
  Synthesized
MNTKYNKEFLLYLAGFVDSDGSIFARIEPTQSAKFKHKLRLTFRVWQKTQRRWFLDKLVDEIGVGYVYDTGSVSDYTLSQIKPLHNFLTQLQPFLKLKQKQANLVLKIIEQLPSAKESPDKFLEVCTWVDQIAALNDSKTRKTTSETVRAVLDSLPGSVGGLSPSQASSAASSASSSPGSGISEALRAGAGSGTGYNKEFLLYLAGFVDGDGSIYACILPNQGSKFKHALQLFFTVGQKTCRRWFLDKLVDEIGVGYVHDHGTISQYRLSEIKPLHNFLTQLQPFLKLKQKQANLVLKIIEQLPSAKESPDKFLEVCTWVDQIAALNDSRTRKTTSETVRAVLDSLSEKKKSSP

SEQ ID NO: 13 - protein, 147 aa, Artificial Sequence
  Synthesized
KEFLLYLAGFVDSDGSIFARIEPTQSAKFKHKLRLTFRVHQKTQRRWFLDKLVDEIGVGYVYDTGSVSDYTLSQIKPLHNFLTQLQPFLKLKQKQANLVLKIIEQLPSAKESPDKFLEVCTWVDQIAALNDSKTRKTTSETVRAVLD

SEQ ID NO: 14 - protein, 147 aa, Artificial Sequence
  Synthesized
KEFLLYLAGFVDADGSIFARIEPTQSAKFKHKLRLTFRVHQKTQRRWFLDKLVDEIGVGYVYDTGSVSDYTLSEIKPLHNFLTQLQPFLKLKQKQANLVLKIIEQLPSAKESPDKFLEVCTWVDQIAALNDSKTRKTTSETVRAVLD

SEQ ID NO: 15 - protein, 147 aa, Artificial Sequence
  Synthesized
KEFLLYLAGFVDADGSIFARIEPTQSAKFKHKLRLTFRVHQKTQRRWFLDKLVDEIGVGYVYDTGSVSDYTLSQIKPLHNFLTQLQPFLKLKQKQANLVLKIIEQLPSAKESPDKFLEVCTWVDQIAALNDSKTRKTTSETVRAVLD

SEQ ID NO: 16 - protein, 147 aa, Artificial Sequence; identical to SEQ ID NO: 14
  Synthesized

SEQ ID NO: 17 - protein, 147 aa, Artificial Sequence; identical to SEQ ID NO: 15
  Synthesized

SEQ ID NO: 18 - protein, 147 aa, Artificial Sequence
  Synthesized
KEFLLYLAGFVDADGSIFARIEPTQSAKFKHKLRLTFRVWQKTQRRWFLDKLVDEIGVGYVYDEGSVSSYTLSEIKPLHNFLTQLQPFLKLKQKQANLVLKIIEQLPSAKESPDKFLEVCTWVDQIAALNDSKTRKTTSETVRAVLD

SEQ ID NO: 19 - protein, 147 aa, Artificial Sequence; identical to SEQ ID NO: 13
  Synthesized

SEQ ID NO: 20 - protein, 147 aa, Artificial Sequence
  Synthesized
KEFLLYLAGFVDSDGSIFARIEPTQSAKFKHKLRLTFRVWQKTQRRWFLDKLVDEIGVGYVYDEGSVSSYTLSEIKPLHNFLTQLQPFLKLKQKQANLVLKIIEQLPSAKESPDKFLEVCTWVDQIAALNDSKTRKTTSETVRAVLD

SEQ ID NO: 21 - protein, 147 aa, Artificial Sequence; identical to SEQ ID NO: 13
  Synthesized

SEQ ID NO: 22 - protein, 147 aa, Artificial Sequence
  Synthesized
KEFLLYLAGFVDSDGSIFARIEPTQSAKFKHKLRLTFRVWQKTQRRWFLDKLVDEIGVGYVYDTGSVSDYTLSQIKPLHNFLTQLQPFLKLKQKQANLVLKIIEQLPSAKESPDKFLEVCTWVDQIAALNDSKTRKTTSETVRAVLD

SEQ ID NO: 23 - protein, 147 aa, Artificial Sequence
  Synthesized
KEFLLYLAGFVDGDGSIYACILPNQGSKFKHALQLFFTVGQKTCRRWFLDKLVDEIGVGYVHDHGTISQYRLSEIKPLHNFLTQLQPFLKLKQKQANLVLKIIEQLPSAKESPDKFLEVCTWVDQIAALNDSRTRKTTSETVRAVLD

SEQ ID NO: 24 - protein, 147 aa, Artificial Sequence
  Synthesized
KEFLLYLAGFVDGDGSIYACILPNQGSKFKHALQLFFTVGQKTCRRWFLDKLVDEIGVGYVNDFGSISQYRLSEIKPLYNFLTQLQPFLKLKQKQANLVLKIIEQLPSAKESPDKFLEVCTWVDQIAALNDSRTRKTTSETVRAVLD

SEQ ID NO: 25 - protein, 147 aa, Artificial Sequence
  Synthesized
KEFLLYLAGFVDGDGSIYACILPNQGSKFKHALQLFFTVGQKTCRRWFLDKLVDEIGVGYVHDFGLISQYRLSEIKPLHNFLTQLQPFLKLKQKQANLVLKIIEQLPSAKESPDKFLEVCTWVDQIAALNDSRTRKTTSETVRAVLD

SEQ ID NO: 26 - protein, 147 aa, Artificial Sequence
  Synthesized
KEFLLYLAGFVDGDGSIYACILPNQGSKFKHALQLFFTVGQKTCRRWFLDKLVDEIGVGYVHDHGLIAQYRLSEIKPLHNFLTQLQPFLKLKQKQANLVLKIIEQLPSAKESPDKFLEVCTWVDQIAALNDSRTRKTTSETVRAVLD

SEQ ID NO: 27 - protein, 147 aa, Artificial Sequence
  Synthesized
KEFLLYLAGFVDGDGSIYACILPNQGSKFKHALQLFFTVGQKTCRRWFLDKLVDEIGVGYVNDFGPVSQYRLSEIKPLHNFLTQLQPFLKLKQKQANLVLKIIEQLPSAKESPDKFLEVCTWVDQIAALNDSRTRKTTSETVRAVLD

SEQ ID NO: 28 - protein, 147 aa, Artificial Sequence
  Synthesized
KEFLLYLAGFVDGDGSIYACILPNQGSKFKHALQLFFTVGQKTCRRWFLDKLVDEIGVGYVQDHGRISQYRLSEIKPLHNFLTQLQPFLKLKQKQANLVLKIIEQLPSAKESPDKFLEVCTWVDQIAALNDSRTRKTTSETVRAVLD

SEQ ID NO: 29 - protein, 147 aa, Artificial Sequence
  Synthesized
KEFLLYLAGFVDGDGSIYACILPNQGSKFKHALQLFFTVGQKTCRRWFLDKLVDEIGVGYVQDHGTISQYRLSEIKPLHNFLTQLQPFLKLKQKQANLVLKIIEQLPSAKESPDKFLEVCTWVDQIAALNDSRTRKTTSETVRAVLD

SEQ ID NO: 30 - protein, 147 aa, Artificial Sequence; identical to SEQ ID NO: 28
  Synthesized

SEQ ID NO: 31 - protein, 147 aa, Artificial Sequence
  Synthesized
KEFLLYLAGFVDGDGSIYACILPNQGSKFKHALQLFFTVGQKTCRRWFLDKLVDEIGVGYVHDHGRISQYRLSEIKPLHNFLTQLQPFLKLKQKQANLVLKIIEQLPSAKESPDKFLEVCTWVDQIAALNDSRTRKTTSETVRAVLD

SEQ ID NO: 32 - protein, 147 aa, Artificial Sequence; identical to SEQ ID NO: 23
  Synthesized

SEQ ID NO: 33 - DNA, 1062 bp, Artificial Sequence
  Synthesized
atgaatacaaaatataataaagagttcttactctacttagcagggtttgtagactctgacggttccatctttgcccgtatcgagcctactcaaagtgctaagttcaagcacaagctgaggctcacgttccgggtccatcagaagacacagcgccgttggttcctcgacaagctggtggacgagatcggtgtgggttacgtgtatgacactggcagcgtctccgattacactctgtcccagatcaagcctttgcataattttttaacacaactacaaccttttctaaaactaaaacaaaaacaagcaaatttagttttaaaaattattgaacaacttccgtcagcaaaagaatccccggacaaattcttagaagtttgtacatgggtggatcaaattgcagctctgaatgattcgaagacgcgtaaaacaacttctgaaaccgttcgtgctgtgctagacagtttaccaggatccgtgggaggtctatcgccatctcaggcatccagcgccgcatcctcggcttcctcaagcccgggttcagggatctccgaagcactcagagctggagcaggttccggcactggatacaacaaggaattcctgctctacctggcgggcttcgtcgacggggacggctccatctatgcctgtatccttcctaatcaagggagtaagttcaagcacgctctgcagctctttttcacggtcggccagaagacatgccgccgttggttcctcgacaagctggtggacgagatcggtgtgggttacgtgcacgaccacggcactatctcgcagtaccgcctgtccgagatcaagcctctgcacaacttcctgacccagctccagcccttcctgaagctcaagcagaagcaggccaacctcgtgctgaagatcatcgagcagctgccctccgccaaggaatccccggacaagttcctggaggtgtgcacctgggtggaccagatcgccgctctgaacgactccaggacccgcaagaccacttccgaaaccgtccgcgccgttctagacagtctctccgagaagaagaagtcgtccccc

SEQ ID NO: 34 - DNA, 1062 bp, Artificial Sequence
  Synthesized
atgaatacaaaatataataaagagttcttactctacttagcagggtttgtagacgctgacggttccatctttgcccgtatcgagcctactcaaagtgctaagttcaagcacaagctgaggctcacgttccgggtccatcagaagacacagcgccgttggttcctcgacaagctggtggacgagatcggtgtgggttacgtgtatgacactggcagcgtctccgattacactctgtccgagatcaagcctttgcataattttttaacacaactacaaccttttctaaaactaaaacaaaaacaagcaaatttagttttaaaaattattgaacaacttccgtcagcaaaagaatccccggacaaattcttagaagtttgtacatgggtggatcaaattgcagctctgaatgattcgaagacgcgtaaaacaacttctgaaaccgttcgtgctgtgctagacagtttaccaggatccgtgggaggtctatcgccatctcaggcatccagcgccgcatcctcggcttcctcaagcccgggttcagggatctccgaagcactcagagctggagcaggttccggcactggatacaacaaggaattcctgctctacctggcgggcttcgtcgacggggacggctccatctatgcctgtatccttcctaatcaagggagtaagttcaagcacgctctgcagctctttttcacggtcggccagaagacatgccgccgttggttcctcgacaagctggtggacgagatcggtgtgggttacgtgaacgacttcggctctatctcgcagtaccgcctgtccgagatcaagcctctgtacaacttcctgacccagctccagcccttcctgaagctcaagcagaagcaggccaacctcgtgctgaagatcatcgagcagctgccctccgccaaggaatccccggacaagttcctggaggtgtgcacctgggtggaccagatcgccgctctgaacgactccaggacccgcaagaccacttccgaaaccgtccgcgccgttctagacagtctctccgagaagaagaagtcgtccccc

SEQ ID NO: 35 - DNA, 1062 bp, Artificial Sequence
  Synthesized
atgaatacaaaatataataaagagttcttactctacttagcagggtttgtagacgctgacggttccatctttgcccgtatcgagcctactcaaagtgctaagttcaagcacaagctgaggctcacgttccgggtccatcagaagacacagcgccgttggttcctcgacaagctggtggacgagatcggtgtgggttacgtgtatgacactggcagcgtctccgattacactctgtcccagatcaagcctttgcataattttttaacacaactacaaccttttctaaaactaaaacaaaaacaagcaaatttagttttaaaaattattgaacaacttccgtcagcaaaagaatccccggacaaattcttagaagtttgtacatgggtggatcaaattgcagctctgaatgattcgaagacgcgtaaaacaacttctgaaaccgttcgtgctgtgctagacagtttaccaggatccgtgggaggtctatcgccatctcaggcatccagcgccgcatcctcggcttcctcaagcccgggttcagggatctccgaagcactcagagctggagcaggttccggcactggatacaacaaggaattcctgctctacctggcgggcttcgtcgacggggacggctccatctatgcctgtatccttcctaatcaagggagtaagttcaagcacgctctgcagctctttttcacggtcggccagaagacatgccgccgttggttcctcgacaagctggtggacgagatcggtgtgggttacgtgcacgacttcggcctgatctcgcagtaccgcctgtccgagatcaagcctctgcacaacttcctgacccagctccagcccttcctgaagctcaagcagaagcaggccaacctcgtgctgaagatcatcgagcagctgccctccgccaaggaatccccggacaagttcctggaggtgtgcacctgggtggaccagatcgccgctctgaacgactccaggacccgcaagaccacttccgaaaccgtccgcgccgttctagacagtctctccgagaagaagaagtcgtccccc

SEQ ID NO: 36 - DNA, 1062 bp, Artificial Sequence
  Synthesized
atgaatacaaaatataataaagagttcttactctacttagcagggtttgtagacgctgacggttccatctttgcccgtatcgagcctactcaaagtgctaagttcaagcacaagctgaggctcacgttccgggtccatcagaagacacagcgccgttggttcctcgacaagctggtggacgagatcggtgtgggttacgtgtatgacactggcagcgtctccgattacactctgtccgagatcaagcctttgcataattttttaacacaactacaaccttttctaaaactaaaacaaaaacaagcaaatttagttttaaaaattattgaacaacttccgtcagcaaaagaatccccggacaaattcttagaagtttgtacatgggtggatcaaattgcagctctgaatgattcgaagacgcgtaaaacaacttctgaaaccgttcgtgctgtgctagacagtttaccaggatccgtgggaggtctatcgccatctcaggcatccagcgccgcatcctcggcttcctcaagcccgggttcagggatctccgaagcacccagagctggagcaggttccggcactggatacaacaaggaattcctgctctacctggcgggcttcgtcgacggggacggctccatctatgcctgtatccttcctaatcaagggagtaagttcaagcacgctctgcagctctttttcacggtcggccagaagacatgccgccgttggttcctcgacaagctggtggacgagatcggtgtgggttacgtgcacgaccacggccttatcgcgcagtaccgcctgtccgagatcaagcctctgcacaacttcctgacccagctccagcccttcctgaagctcaagcagaagcaggccaacctcgtgctgaagatcatcgagcagctgccctccgccaaggaatccccggacaagttcctggaggtgtgcacctgggtggaccagatcgccgctctgaacgactccaggacccgcaagaccacttccgaaaccgtccgcgccgttctagacagtctctccgagaagaagaagtcgtccccc

SEQ ID NO: 37 - DNA, 1062 bp, Artificial Sequence
  Synthesized
atgaatacaaaatataataaagagttcttactctacttagcagggtttgtagacgctgacggttccatctttgcccgtatcgagcctactcaaagtgctaagttcaagcacaagctgaggctcacgttccgggtccatcagaagacacagcgccgttggttcctcgacaagctggtggacgagatcggtgtgggttacgtgtatgacactggcagcgtctccgattacactctgtcccagatcaagcctttgcataattttttaacacaactacaaccttttctaaaactaaaacaaaaacaagcaaatttagttttaaaaattattgaacaacttccgtcagcaaaagaatccccggacaaattcttagaagtttgtacatgggtggatcaaattgcagctctgaatgattcgaagacgcgtaaaacaacttctgaaactgttcgtgctgtgctagacagtttaccaggatccgtgggaggtctatcgccatctcaggcatccagcgccgcatcctcggcttcctcaagcccgggttcagggatctccgaagcactcagagctggagcaggttccggcactggatacaacaaggaattcctgctctacctggcgggcttcgtcgacggggacggctccatctatgcctgtatccttcctaatcaagggagtaagttcaagcacgctctgcagctctttttcacggtcggccagaagacatgccgccgttggttcctcgacaagctggtggacgagatcggtgtgggttacgtgaacgacttcggccctgtctcgcagtaccgcctgtccgagatcaagcctctgcacaacttcctgacccagctccagcccttcctgaagctcaagcagaagcaggccaacctcgtgctgaagatcatcgagcagctgccctccgccaaggaatccccggacaagttcctggaggtgtgcacctgggtggaccagatcgccgctctgaacgactccaggacccgcaagaccacttccgaaaccgtccgcgccgttctagacagtctctccgagaagaagaagtcgtccccc

SEQ ID NO: 38 - DNA, 1062 bp, Artificial Sequence
  Synthesized
atgaatacaaaatataataaagagttcttactctacttagcagggtttgtagacgctgacggttccatctttgcccgtatcgagcctactcaaagtgctaagttcaagcacaagctgaggctcacgttccgggtctggcagaagacacagcgccgttggttcctcgacaagctggtggacgagatcggtgtgggttacgtgtatgacgagggcagcgtctcctcttacactctgtccgagatcaagcctttgcataattttttaacacaactacaaccttttctaaaactaaaacaaaaacaagcaaatttagttttaaaaattattgaacaacttccgtcagcaaaagaatccccggacaaattcttagaagtttgtacatgggtggatcaaattgcagctctgaatgattcgaagacgcgtaaaacaacttctgaaaccgttcgtgctgtgctagacagtttaccaggatccgtgggaggtctatcgccatctcaggcatccagcgccgcatcctcggcttcctcaagcccgggttcagggatctccgaagcactcagagctggagcaggttccggcactggatacaacaaggaattcctgctctacctggcgggcttcgtcgacggggacggctccatctatgcctgtatccttcctaatcaagggagtaagttcaagcacgctctgcagctattcttcacggtcggccagaagacatgccgccgttggttcctcgacaagctggtggacgagatcggtgtgggttacgtgcaggaccacggcaggatctcgcagtaccgcctgtccgagatcaagcctctgcacaacttcctgacccagctccagcccttcctgaagctcaagcagaagcaggccaacctcgtgctgaagatcatcgagcagctgccctccgccaaggaatccccggacaagttcctggaggtgtgcacctgggtggaccagatcgccgctctgaacgactccaggacccgcaagaccacttccgaaaccgtccgcgccgttctagacagtctctccgagaagaagaagtcgtccccc

SEQ ID NO: 39 - DNA, 1062 bp, Artificial Sequence
  Synthesized
atgaatacaaaatataataaagagttcttactctacttagcagggtttgtagactctgacggttccatctttgcccgtatcgagcctactcaaagtgctaagttcaagcacaagctgaggctcacgttccgggtccatcagaagacacagcgccgttggttcctcgacaagctggtggacgagatcggtgtgggttacgtgtatgacactggcagcgtctccgattacactctgtcccagatcaagcctttgcataattttttaacacaactacaaccttttctaaaactaaaacaaaaacaagcaaatttagttttaaaaattattgaacaacttccgtcagcaaaagaatccccggacaaattcttagaagtttgtacatgggtggatcaaattgcagctctgaatgattcgaagacgcgtaaaacaacttctgaaaccgttcgtgctgtgctagacagtttaccaggatccgtgggaggtctatcgccatctcaggcatccagcgccgcatcctcggcttcctcaagcccgggttcagggatctccgaagcactcagagctggagcaggttccggcactggatacaacaaggaattcctgctctacctggcgggcttcgtcgacggggacggctccatctatgcctgtatccttcctaatcaagggagtaagttcaagcacgctctgcagctctttttcacggtcggccagaagacatgccgccgttggttcctcgacaagctggtggacgagatcggtgtgggttacgtgcaggaccacggcactatctcgcagtaccgcctgtccgagatcaagcctctgcacaacttcctgacccagctccagcccttcctgaagctcaagcagaagcaggccaacctcgtgctgaagatcatcgagcagctgccctccgccaaggaatccccggacaagttcctggaggtgtgcacctgggtggaccagatcgccgctctgaacgactccaggacccgcaagaccacttccgaaaccgtccgcgccgttctagacagtctctccgagaagaagaagtcgtccccc

SEQ ID NO: 40 - DNA, 1062 bp, Artificial Sequence
  Synthesized
atgaatacaaaatataataaagagttcttactctacttagcagggtttgtagactctgacggttccatctttgcccgtatcgagcctactcaaagtgctaagttcaagcacaagctgaggctcacgttccgggtctggcagaagacacagcgccgttggttcctcgacaagctggtggacgagatcggtgtgggttacgtgtatgacgagggcagcgtctcctcttacactctgtccgagatcaagcctttgcataattttttaacacaactacaaccttttctaaaactaaaacaaaaacaagcaaatttagttttaaaaattattgaacaacttccgtcagcaaaagaatccccggacaaattcttagaagtttgtacatgggtggatcaaattgcagctctgaatgattcgaagacgcgtaaaacaacttctgaaaccgttcgtgctgtgctagacagtttaccaggatccgtgggaggtctatcgccatctcaggcatccagcgccgcatcctcggcttcctcaagcccgggttcagggatctccgaagcactcagagctggagcaggttccggcactggatacaacaaggaattcctgctctacctggcgggcttcgtcgacggggacggctccatctatgcctgtatccttcctaatcaagggagtaagttcaagcacgctctgcagctattcttcacggtcggccagaagacatgccgccgttggttcctcgacaagctggtggacgagatcggtgtgggttacgtgcaggaccacggcaggatctcgcagtaccgcctgtccgagatcaagcctctgcacaacttcctgacccagctccagcccttcctgaagctcaagcagaagcaggccaacctcgtgctgaagatcatcgagcagctgccctccgccaaggaatccccggacaagttcctggaggtgtgcacctgggtggaccagatcgccgctctgaacgactccaggacccgcaagaccacttccgaaaccgtccgcgccgttctagacagtctctccgagaagaagaagtcgtccccc

SEQ ID NO: 41 - DNA, 1062 bp, Artificial Sequence
  Synthesized
atgaatacaaaatataataaagagttcttactctacttagcagggtttgtagactctgacggttccatctttgcccgtatcgagcctactcaaagtgctaagttcaagcacaagctgaggctcacgttccgggtccatcagaagacacagcgccgttggttcctcgacaagctggtggacgagatcggtgtgggttacgtgtatgacactggcagcgtctccgattacactctgtcccagatcaagcctttgcataattttttaacacaactacaaccttttctaaaactaaaacaaaaacaagcaaatttagttttaaaaattattgaacaacttccgtcagcaaaagaatccccggacaaattcttagaagtttgtacatgggtggatcaaattgcagctctgaatgattcgaagacgcgtaaaacaacttctgaaaccgttcgtgctgtgctagacagtttaccaggatccgtgggaggtctatcgccatctcaggcatccagcgccgcatcctcggcttcctcaagcccgggttcagggatctccgaagcactcagagctggagcaggttccggcactggatacaacaaggaattcctgctctacctggcgggcttcgtcgacggggacggctccatctatgcctgtatccttcctaatcaagggagtaagttcaagcacgctctgcagctctttttcacggtcggccagaagacatgccgccgttggttcctcgacaagctggtggacgagatcggtgtgggttacgtgcacgaccacggcaggatctcgcagtaccgcctgtccgagatcaagcctctgcacaacttcctgacccagctccagcccttcctgaagctcaagcagaagcaggccaacctcgtgctgaagatcatcgagcagctgccctccgccaaggaatccccggacaagttcctggaggtgtgcacctgggtggaccagatcgccgctctgaacgactccaggacccgcaagaccacttccgaaaccgtccgcgccgttctagacagtctctccgagaagaagaagtcgtccccc

SEQ ID NO: 42 - DNA, 1062 bp, Artificial Sequence
  Synthesized
atgaatacaaaatataataaagagttcttactctacttagcagggtttgtagactctgacggttccatctttgcccgtatcgagcctactcaaagtgctaagttcaagcacaagctgaggctcacgttccgggtctggcagaagacacagcgccgttggttcctcgacaagctggtggacgagatcggtgtgggttacgtgtatgacactggcagcgtctccgattacactctgtcccagatcaagcctttgcataattttttaacacaactacaaccttttctaaaactaaaacaaaaacaagcaaatttagttttaaaaattattgaacaacttccgtcagcaaaagaatccccggacaaattcttagaagtttgtacatgggtggatcaaattgcagctctgaatgattcgaagacgcgtaaaacaacttctgaaaccgttcgtgctgtgctagacagtttaccaggatccgtgggaggtctatcgccatctcaggcatccagcgccgcatcctcggcttcctcaagcccgggttcagggatctccgaagcactcagagctggagcaggttccggcactggatacaacaaggaattcctgctctacctggcgggcttcgtcgacggggacggctccatctatgcctgtatccttcctaatcaagggagtaagttcaagcacgctctgcagctctttttcacggtcggccagaagacatgccgccgttggttcctcgacaagctggtggacgagatcggtgtgggttacgtgcacgaccacggcactatctcgcagtaccgcctgtccgagatcaagcctctgcacaacttcctgacccagctccagcccttcctgaagctcaagcagaagcaggccaacctcgtgctgaagatcatcgagcagctgccctccgccaaggaatccccggacaagttcctggaggtgtgcacctgggtggaccagatcgccgctctgaacgactccaggacccgcaagaccacttccgaaaccgtccgcgccgttctagacagtctctccgagaagaagaagtcgtccccc

SEQ ID NO: 43 - protein, 35 aa, Homo sapiens
MSVLTPLLLRGLTGSARRLPVPRAKIHSLPPEGKL

SEQ ID NO: 44 - protein, 63 aa, Neurospora crassa
MASTRVLASRLASQMAASAKVARPAVRVAQVSKRTIQTGSPLQTLKRTQMTSIVNATTRQAFQ

SEQ ID NO: 45 - protein, 98 aa, Artificial Sequence
  Synthesized
MSVLTPLLLRGLTGSARRLPVPRAKIHSLPPEGKLMASTRVLASRLASQMAASAKVARPAVRVAQVSKRTIQTGSPLQTLKRTQMTSIVNATTRQAFQ

SEQ ID NO: 46 - protein, 18 aa, Mouse parovirus NS2
VDEMTKKFGTLTIHDTEK

SEQ ID NO: 47 - protein, 10 aa, Artificial Sequence
  Synthesized
LGAGLGALGL

SEQ ID NO: 48 - protein, 163 aa, Chlamydomonas reinhardtii
MNTKYNKEFLLYLAGFVDGDGSIIAQIKPNQSYKFKHQLSLAFQVTQKTQRRWFLDKLVDEIGVGYVRDRGSVSDYILSEIKPLHNFLTQLQPFLKLKQKQANLVLKIIWRLPSAKESPDKFLEVCTWVDQIAALNDSKTRKTTSETVRAVLDSLSEKKKSSP

SEQ ID NO: 49 - DNA, 20 bp, Artificial Sequence
  Synthesized
agccccgggtactccttgtt

SEQ ID NO: 50 - DNA, 18 bp, Artificial Sequence
  Synthesized
ttccttgcaggaacagag

SEQ ID NO: 51 - DNA, 17 bp, Artificial Sequence
  Synthesized
ctgcttgaccacccatt

SEQ ID NO: 52 - DNA, 19 bp, Artificial Sequence
  Synthesized
ccagcaggccaggtacacc

SEQ ID NO: 53 - DNA, 16 bp, Artificial Sequence
  Synthesized
accgccaaggatgcac

SEQ ID NO: 54 - DNA, 16 bp, Artificial Sequence
  Synthesized
gcgggtgggaatggag

SEQ ID NO: 55 - DNA, 27 bp, Artificial Sequence
  Synthesized
gctggctagcgtttaaacttaagcttg

SEQ ID NO: 56 - DNA, 34 bp, Artificial Sequence
  Synthesized
gggtatgttgttaagaagaggaattgaacctctg

SEQ ID NO: 57 - DNA, 31 bp, Artificial Sequence
  Synthesized
tgtgagtgcatataatgaaatgggatgacag

SEQ ID NO: 58 - DNA, 29 bp, Artificial Sequence
  Synthesized
cagtccccacctcttaagtttcaaatgac

SEQ ID NO: 59 - DNA, 20 bp, Artificial Sequence
  Synthesized
ccgcaagccccttggtactg

SEQ ID NO: 60 - DNA, 23 bp, Artificial Sequence
  Synthesized
gtctgcactcaaggaaggagctc

SEQ ID NO: 61 - DNA, 32 bp, Artificial Sequence
  Synthesized
gaccttatgctgaggaaaagctgtcattctag

SEQ ID NO: 62 - DNA, 32 bp, Artificial Sequence
  Synthesized
ggccatttatttcagagtttagatcgctatgc

SEQ ID NO: 63 - DNA, 14 bp, Artificial Sequence
  Synthesized
tggcagggcccggt

SEQ ID NO: 64 - DNA, 22 bp, Artificial Sequence
  Synthesized
cccaagaacagggtttgttaag

SEQ ID NO: 65 - DNA, 19 bp, Artificial Sequence
  Synthesized
ggaatgccattgcgattag

SEQ ID NO: 66 - DNA, 26 bp, Artificial Sequence
  Synthesized
agcagttctaccgtacaaccctaaca

SEQ ID NO: 67 - DNA, 18 bp, Artificial Sequence
  Synthesized
ggcagttgaggtggatta

SEQ ID NO: 68 - DNA, 20 bp, Artificial Sequence
  Synthesized
ggaatgcggtagtagttagg

SEQ ID NO: 69 - DNA, 24 bp, Artificial Sequence
  Synthesized
aaccagacaaatcgctccaccaac

SEQ ID NO: 70 - DNA, 19 bp, Artificial Sequence
  Synthesized
cggacaggattgacagatt

SEQ ID NO: 71 - DNA, 20 bp, Artificial Sequence
  Synthesized
ccagagtctcgttcgttatc

SEQ ID NO: 72 - DNA, 15 bp, Artificial Sequence
  Synthesized
accgggctctgccat